European Patent Application EP 4 435 117 A1, published September 25, 2024. Title: NOVEL METHOD FOR ISOTHERMAL AMPLIFICATION OF PADLOCK PROBES FOR NUCLEIC ACID DETECTION AND PHI29 DNA POLYMERASE VARIANTS. Applicant: Consejo Superior de Investigaciones Científicas (CSIC). The sequence listing filed with the application follows.

SEQUENCE LISTING (27 sequences)

SEQ ID NO: 1 - protein, 685 aa, synthetic construct
MPRKMYSCDFETTTKVEDCRVWAYGYMNIEDHSEYKIGNSLDEFMAWVLKVQADLYFHNLKFDGAFIINWLERNGFKWSADGLPNTYNTIISRMGQWYMIDICLGYKGKRKIHTVIYDSLKKLPFPVKKIAKDFKLTVLKGDIDYHKERPVGYKITPEEYAYIKNDIQIIAEALLIQFKQGLDRMTAGSDSLKGFKDIITTKKFKKVFPTLSLGLDKEVRYAYRGGFTWLNDRFKEKEIGEGMVFDVNSLYPAQMYSRLLPYGEPIVFEGKYVWDEDYPLHIQHIRCEFELKEGYIPTIQIKRSRFYKGNEYLKSSGGEIADLWLSNVDLELMKEHYDLYNVEYISGLKFKATTGLFKDFIDKWTYIKTTSEGAIKQLAKLMLNSLYGKFASNPDVTGKVPYLKENGALGFRLGEEETKDPVYTPMGVFITAWARYTTITAAQACYDRIIYCDTDSIHLTGTEIPDVIKDIVDPKKLGYWAHESTFKRAKYLRQKTYIQDIYMKEVDGKLVEGSPDDYTDIKFSVKCAGMTDKIKKEVTFENFKVGFSRKMKPKPVQVPGGVVLVDDTFTIKGTGSGAWKEWLERKVGEGRARRLIEYFGSAGEVGKLVENAEVSKLLEVPGIGDEAVARLVPGYKTLRDAGLTPAEAERVLKRYGSVSKVQEGATPDELRELGLGDAKIARILG

SEQ ID NO: 2 - protein, 293 aa, synthetic construct
MRPIEHALSYAAQGYGVLPLRPGGKEPLGKLVPHGLKNASRDPATLEAWWRSCPRCGVGILPGPEVLVLDFDDPEAWEGLRQEHPALEAAPRQRTPKGGRHVFLRLPEGVRLSASVRAIPGVDLRGMGRAYVVAAPTRLKDGRTYTWEAPLTPPEELPPVPQALLLKLLPPPPPPRPSWGAVGTASPKRLQALLQAYAAQVARTPEGQRHLTLIRYAVAAGGLIPHGLDPREAEEVLVAAAMSAGLPEWEARDAVRWGLGVGASRPLVLESSSKPPEPRTYRARVYARMRRWV

SEQ ID NO: 3 - protein, 685 aa, synthetic construct
MPRKMYSCDFETTTKVEDCRVWAYGYMNIEDHSEYKIGNSLDEFMAWVLKVQADLYFHNLKFDGAFIINWLERNGFKWSADGLPNTYNTIISRMGQWYMIDICLGYKGKRKIHTVIYDSLKKLPFPVKKIAKDFKLTVLKGDIDYHKERPVGYKITPEEYAYIKNDIQIIAEALLIQFKQGLDRMTAGSDSLKGFKDIITTKKFKKVFPTLSLGLDKEVRYAYRGGFTWLNDRFKEKEIGEGMVFDVNSLYPAQMYSRLLPYGEPIVFEGKYVWDEDYPLHIQHIRCEFELKEGYIPTIQIKRSRFYKGNEYLKSSGGEIADLWLSNVDLELMKEHYDLYNVEYISGLKFKATTGLFKDFIDKWTYIKTTSEGAIKQLAKLMLNSLYGKFASNPDVTGKVPYLKENGALGFRLGKKKTKDPVYTPMGVFITAWARYTTITAAQACYDRIIYCDTDSIHLTGTEIPDVIKDIVDPKKLGYWAHESTFKRAKYLRQKTYIQDIYMKEVDGKLVEGSPDDYTDIKFSVKCAGMTDKIKKEVTFENFKVGFSRKMKPKPVQVPGGVVLVDDTFTIKGTGSGAWKEWLERKVGEGRARRLIEYFGSAGEVGKLVENAEVSKLLEVPGIGDEAVARLVPGYKTLRDAGLTPAEAERVLKRYGSVSKVQEGATPDELRELGLGDAKIARILG

SEQ ID NO: 4 - protein, 572 aa, synthetic construct
MPRKMYSCDFETTTKVEDCRVWAYGYMNIEDHSEYKIGNSLDEFMAWVLKVQADLYFHNLKFDGAFIINWLERNGFKWSADGLPNTYNTIISRMGQWYMIDICLGYKGKRKIHTVIYDSLKKLPFPVKKIAKDFKLTVLKGDIDYHKERPVGYKITPEEYAYIKNDIQIIAEALLIQFKQGLDRMTAGSDSLKGFKDIITTKKFKKVFPTLSLGLDKEVRYAYRGGFTWLNDRFKEKEIGEGMVFDVNSLYPAQMYSRLLPYGEPIVFEGKYVWDEDYPLHIQHIRCEFELKEGYIPTIQIKRSRFYKGNEYLKSSGGEIADLWLSNVDLELMKEHYDLYNVEYISGLKFKATTGLFKDFIDKWTYIKTTSEGAIKQLAKLMLNSLYGKFASNPDVTGKVPYLKENGALGFRLGEEETKDPVYTPMGVFITAWARYTTITAAQACYDRIIYCDTDSIHLTGTEIPDVIKDIVDPKKLGYWAHESTFKRAKYLRQKTYIQDIYMKEVDGKLVEGSPDDYTDIKFSVKCAGMTDKIKKEVTFENFKVGFSRKMKPKPVQVPGGVVLVDDTFTIK

SEQ ID NO: 5 - protein, 685 aa, synthetic construct
MPRKMYSCDFETTTKVEDCRVWAYGYMNIEDHSEYKIGNSLDEFMAWVLKVQADLYFHNLKFDGAFIINWLERNGFKWSADGLPNTYNTIISRMGQWYMIDICLGYKGKRKIHTVIYDSLKKLPFPVKKIAKDFKLTVLKGDIDYHKERPVGYKITPEEYAYIKNDIQIIAEALLIQFKQGLDRMTAGSDSLKGFKDIITTKKFKKVFPTLSLGLDKMVRYAYRGGFTWLNDRFKEKEIGEGMVFDVNSLYPAQMYSRLLPYGEPILFEGKYVWDEDYPLHIQHIRCEFELKEGYIPTIQIKRSRFYKGNEYLKSSGGEIADLWLSNVDLELMKEHYDLYNVEYISGLKFKATTGLFKDFIDKWTYIKTTSEGAIKQLAKLMLNSLYGKFASNPDVTGKVPYLKENGALGFRLGKKKTKDPVYTPMGVFITAWARYTTITAAQACYDRIIYCDTDSIHLTGTEIPDVIKDIVDPKKLGYWAHESTFKRAKYLRQKTYIQDIYMKEVDGKLVEGSPDDYTDIKFSVKCAGMTDKIKKEVTFENFKVGFSRKMKPKPVQVPGGVVLVDDTFTIKGTGSGAWKEWLERKVGEGRARRLIEYFGSAGEVGKLVENAEVSKLLEVPGIGDEAVARLVPGYKTLRDAGLTPAEAERVLKRYGSVSKVQEGATPDELRELGLGDAKIARILG

SEQ ID NO: 6 - protein, 298 aa, synthetic construct
MAITKPLLAATLENIEDVQFPCLATPKIDGIRSVKQTQMLSRTFKPIRNSVMNRLLTELLPEGSDGEISIEGATFQDTTSAVMTGHKMYNAKFSYYWFDYVTDDPLKKYIDRVEDMKNYITVHPHILEHAQVKIIPLIPVEINNITELLQYERDVLSKGFEGVMIRKPDGKYKFGRSTLKEGILLKMKQFKDAEATIISMTALFKNTNTKTKDNFGYSKRSTHKSGKVEEDVMGSIEVDYDGVVFSIGTGFDADQRRDFWQNKESYIGKMVKFKYFEMGSKDCPRFPVFIGIRHEEDR

SEQ ID NO: 7 - DNA, 75 bp, synthetic construct
  source 1..75: mol_type = other DNA
tgcggtggacgatggaaaaatgtaaaacgacggccgaattcatagctgtttcctgaaaaaccgcctagaagcatt

SEQ ID NO: 8 - DNA, 31 bp, synthetic construct
  source 1..31: mol_type = other DNA
tgcggtggacgatggnccgcctagaagcatt

SEQ ID NO: 9 - DNA, 174 bp, synthetic construct
  source 1..174: mol_type = other DNA
ttcttgaactgttgcgaattcggtaaaacgaccatagctgttgtaaaacgaccatagctgttgtaaaacgaccatagctgttgtaaaacgacctcagccgaccatagctgttgtaaaacgaccatagctgttgtaaaacgaccatagctgttcgatatctgcctggagttgaat

SEQ ID NO: 10 - DNA, 31 bp, synthetic construct
  source 1..31: mol_type = other DNA
ttcttgaactgttgcntgcctggagttgaat

SEQ ID NO: 11 - DNA, 89 bp, synthetic construct
  source 1..89: mol_type = other DNA
aagaagctattaaaatcaccgcaactgaactacttgtcgcctcagcgcatctcctgatgaggttccacctgcctcagcgtcattctcct

SEQ ID NO: 12 - DNA, 31 bp, synthetic construct
  source 1..31: mol_type = other DNA
  variation 20: note = N represents the nucleotide sequence of the backbone region of the padlock probe
aagaagctattaaaatcacngtcattctcct

SEQ ID NO: 13 - DNA, 89 bp, synthetic construct
  source 1..89: mol_type = other DNA
aagaagctattaaaatcaccgcaactgaggtacttgtcgccacagagcatcacctgatgaggttccacctgccacagagtcattctcct

SEQ ID NO: 14 - DNA, 31 bp, synthetic construct; identical to SEQ ID NO: 12
  source 1..31: mol_type = other DNA
  variation 20: note = N represents the nucleotide sequence of the backbone region of the padlock probe

SEQ ID NO: 15 - DNA, 45 bp, synthetic construct
  source 1..45: mol_type = other DNA
tccacctgccacagagtcattctcctaagaagctattaaaatcac

SEQ ID NO: 16 - DNA, 15 bp, synthetic construct
  source 1..15: mol_type = other DNA
tgtaaaacgacggcc

SEQ ID NO: 17 - DNA, 15 bp, synthetic construct
  source 1..15: mol_type = other DNA
caggaaacagctatg

SEQ ID NO: 18 - DNA, 50 bp, synthetic construct
  source 1..50: mol_type = other DNA
tccggcccctccatcgtccaccgcaaatgcttctaggcggactatgactt

SEQ ID NO: 19 - DNA, 10 bp, synthetic construct
  source 1..10: mol_type = other DNA
gtaaaacgac

SEQ ID NO: 20 - DNA, 10 bp, synthetic construct
  source 1..10: mol_type = other DNA
aacagctatg

SEQ ID NO: 21 - DNA, 28 bp, synthetic construct
  source 1..28: mol_type = other DNA
agaagtgtatctcgtactcactgtgatc

SEQ ID NO: 22 - DNA, 15 bp, synthetic construct
  source 1..15: mol_type = other DNA
gatcacagtgagtac

SEQ ID NO: 23 - RNA, 15 nt, synthetic construct
  source 1..15: mol_type = other RNA
gatcacagtgagtac

SEQ ID NO: 24 - RNA, 45 nt, synthetic construct
  source 1..45: mol_type = other RNA
atccccatgtgattttaatagcttcttaggagaatgacaaaaaaa

SEQ ID NO: 25 - RNA, 30 nt, synthetic construct
  source 1..30: mol_type = other RNA
gtgattttaatagcttcttaggagaatgac

SEQ ID NO: 26 - RNA, 37 nt, synthetic construct
  source 1..37: mol_type = other RNA
gtgattttaatagcttcttaggagaatgacaaaaaaa

SEQ ID NO: 27 - RNA, 46 nt, synthetic construct
  source 1..46: mol_type = other RNA
acgtagtcgcaacagttcaagaaattcaactccaggcaagcagtag